European Patent Specification EP 4 048 301 B1, published September 18, 2024. Title: Chimeric polypeptide for regulating immune cells. Applicant: Stichting Het Nederlands Kanker Instituut- Antoni van Leeuwenhoek Ziekenhuis. The sequence listing filed with the application follows.

SEQUENCE LISTING (68 sequences)

SEQ ID NO: 1 - protein, 113 aa, Homo sapiens
RVKFSRSADAPAYQQGQNQLYNELNLGRREEYDVLDKRRGRDPEMGGKPQRRKNPQEGLYNELQKDKMAEAYSEIGMKGERRRGKGHDGLYQGLSTATKDTYDALHMQALPPR

SEQ ID NO: 2 - protein, 55 aa, Homo sapiens
KNRKAKAKPVTRGAGAGGRQRGQNKERPPPVPNPDYEPIRKGQRDLYSGLNQRRI

SEQ ID NO: 3 - protein, 45 aa, Homo sapiens
GHETGRLSGAADTQALLRNDQVYQPLRDRDDAQYSHLGGNWARNK

SEQ ID NO: 4 - protein, 45 aa, Homo sapiens
GQDGVRQSRASDKQTLLPNDQLYQPLKDREDDQYSHLQGNQLRRN

SEQ ID NO: 5 - protein, 42 aa, Homo sapiens
RLKIQVRKAAITSYEKSDGVYTGLSTRNQETYETLKHEKPPQ

SEQ ID NO: 6 - protein, 52 aa, Homo sapiens
YFLGRLVPRGRGAAEAATRKQRITETESPYQELQGQRSDVYSDLNTQRPYYK

SEQ ID NO: 7 - protein, 93 aa, Homo sapiens
FFYGSISRAEAEEHLKLAGMADGLFLLRQCLRSLGGYVLSLVHDVRFHHFPIERQLNGTYAIAGGKAHCGPAELCEFYSRDPDGLPCNLRKPC

SEQ ID NO: 8 - protein, 92 aa, Homo sapiens
WYHSSLTREEAERKLYSGAQTDGKFLLRPRKEQGTYALSLIYGKTVYHYLISQDKAGKYCIPEGTKFDTLWQLVEYLKLKADGLIYCLKEAC

SEQ ID NO: 9 - protein, 93 aa, Homo sapiens
FFFGNITREEAEDYLVQGGMSDGLYLLRQSRNYLGGFALSVAHGRKAHHYTIERELNGTYAIAGGRTHASPADLCHYHSQESDGLVCLLKKPF

SEQ ID NO: 10 - protein, 92 aa, Homo sapiens
WFHGKISREESEQIVLIGSKTNGKFLIRARDNNGSYALCLLHEGKVLHYRIDKDKTGKLSIPEGKKFDTLWQLVEHYSYKADGLLRVLTVPC

SEQ ID NO: 11 - protein, 98 aa, Homo sapiens
WFFKNLSRKDAERQLLAPGNTHGSFLIRESESTAGSFSLSVRDFDQNQGEVVKHYKIRNLDNGGFYISPRITFPGLHELVRHYTNASDGLCTRLSRPC

SEQ ID NO: 12 - protein, 264 aa, Homo sapiens
MPDPAAHLPFFYGSISRAEAEEHLKLAGMADGLFLLRQCLRSLGGYVLSLVHDVRFHHFPIERQLNGTYAIAGGKAHCGPAELCEFYSRDPDGLPCNLRKPCNRPSGLEPQPGVFDCLRDAMVRDYVRQTWKLEGEALEQAIISQAPQVEKLIATTAHERMPWYHSSLTREEAERKLYSGAQTDGKFLLRPRKEQGTYALSLIYGKTVYHYLISQDKAGKYCIPEGTKFDTLWQLVEYLKLKADGLIYCLKEACPNSSASNASG

SEQ ID NO: 13 - protein, 287 aa, Homo sapiens
MASSGMADSANHLPFFFGNITREEAEDYLVQGGMSDGLYLLRQSRNYLGGFALSVAHGRKAHHYTIERELNGTYAIAGGRTHASPADLCHYHSQESDGLVCLLKKPFNRPQGVQPKTGPFEDLKENLIREYVKQTWNLQGQALEQAIISQKPQLEKLIATTAHEKMPWFHGKISREESEQIVLIGSKTNGKFLIRARDNNGSYALCLLHEGKVLHYRIDKDKTGKLSIPEGKKFDTLWQLVEHYSYKADGLLRVLTVPCQKIGTQGNVNFGGRPQLPGSHPATWSAG

SEQ ID NO: 14 - protein, 254 aa, Homo sapiens
MGCGCSSHPEDDWMENIDVCENCHYPIVPLDGKGTLLIRNGSEVRDPLVTYEGSNPPASPLQDNLVIALHSYEPSHDGDLGFEKGEQLRILEQSGEWWKAQSLTTGQEGFIPFNFVAKANSLEPEPWFFKNLSRKDAERQLLAPGNTHGSFLIRESESTAGSFSLSVRDFDQNQGEVVKHYKIRNLDNGGFYISPRITFPGLHELVRHYTNASDGLCTRLSRPCQTQKPQKPWWEDEWEVPRETLKLVERLGAG

SEQ ID NO: 15 - protein, 111 aa, Homo sapiens
RRHQGKQNELSDTAGREINLVDAHLKSEQTEASTRQNSQVLLSETGIYDNDPDLCFRMQEGSEVYSNPCLEENKPGIVYASLNHSVIGPNSRLARNVKEAPTEYASICVRS

SEQ ID NO: 16 - protein, 179 aa, Homo sapiens
KRKGRCSVPAFCSSQAEAPADTPEPTAGHTLYSVLSQGYEKLDTPLRPARQQPTPTSDSSSDSNLTTEEDEDRPEVHKPISGRYEVFDQVTQEGAGHDPAPEGQADYDPVTPYVTEVESVVGENTMYAQVFNLQGKTPVSQKEESSATIYCSIRKPQVVPPPQQNDLEIPESPTYENFT

SEQ ID NO: 17 - protein, 97 aa, Homo sapiens
CSRAARGTIGARRTGQPLKEDPSAVPVFSVDYGELDFQWREKTPEPPVPCVPEQTEYATIVFPSGMGTSSPARRGSADGPRSAQPLRPEDGHCSWPL

SEQ ID NO: 18 - protein, 118 aa, Homo sapiens
KCYFLRKAKAKQMPVEMSRPAVPLLNSNNEKMSDPNMEANSHYGHNDDVRNHAMKPINDNKEPLNSDVQYTEVQVSSAESHKDLGKKDTETVYSEVRKAVPDAVESRYSRTEGSLDGT

SEQ ID NO: 19 - protein, 110 aa, Homo sapiens
RIRQKKAQGSTSSTRLHEPEKNAREITQDTNDITYADLNLPKGKKPAPQAAEPNNHTEYASIQTSPQPASEDTLTYADLDMVHLNRTPKQPAPKPEPSFSEYASVQVPRK

SEQ ID NO: 20 - protein, 114 aa, Homo sapiens
KICRKEARKRAAAEQDVPSTLGPISQGHQHECSAGSSQDHPPPGAATYTPGKGEEQELHYASLSFQGLRLWEPADQEAPSTTEYSEIKIHTGQPLRGPGFGLQLEREMSGMVPK

SEQ ID NO: 21 - protein, 89 aa, Homo sapiens
KARRKQAAGRPEKMDDEDPIMGTITSGSRKKPWPDSPGDQASPPGDAPPLEEQKELHYASLSFSEMKSREPKDQEAPSTTEYSEIKTSK

SEQ ID NO: 22 - protein, 94 aa, Homo sapiens
VRSCRKKSARPAAGVGDTGIEDANAVRGSASQGPLTEPWAEDSPPDQPPPASARSSVGEGELQYASLSFQMVKPWDSRGQEATDTEYSEIKIHR

SEQ ID NO: 23 - protein, 673 aa, Artificial Sequence
  chimeric
MPDPAAHLPFFYGSISRAEAEEHLKLAGMADGLFLLRQCLRSLGGYVLSLVHDVRFHHFPIERQLNGTYAIAGGKAHCGPAELCEFYSRDPDGLPCNLRKPCNRPSGLEPQPGVFDCLRDAMVRDYVRQTWKLEGEALEQAIISQAPQVEKLIATTAHERMPWYHSSLTREEAERKLYSGAQTDGKFLLRPRKEQGTYALSLIYGKTVYHYLISQDKAGKYCIPEGTKFDTLWQLVEYLKLKADGLIYCLKEACPNSSASNASGGGSCSRAARGTIGARRTGQPLKEDPSAVPVFSVDYGELDFQWREKTPEPPVPCVPEQTEYATIVFPSGMGTSSPARRGSADGPRSAQPLRPEDGHCSWPLSGGGSDEMEECSQHLPGAGSSGDIMDYKDDDDKGSSGTGSGSGTSAPITAYAQQTRGLLGCIITSLTGRDKNQVEGEVQIVSTATQTFLATCINGVCWAVYHGAGTRTIASPKGPVIQMYTNVDQDLVGWPAPQGSRSLTPCTCGSSDLYLVTRHADVIPVRRRGDSRGSLLSPRPISYLKGSSGGPLLCPAGHAVGLFRAAVCTRGVAKAVDFIPVENLETTMRSPVFTDNSSPPAVTLTHPITKIDTKYIMTCMSADLEVVTSTWVLVGGVLAALAAYCLSTGCVVIVGRIVLSGKPAIIPDREVLY

SEQ ID NO: 24 - protein, 687 aa, Artificial Sequence
  chimeric
MPDPAAHLPFFYGSISRAEAEEHLKLAGMADGLFLLRQCLRSLGGYVLSLVHDVRFHHFPIERQLNGTYAIAGGKAHCGPAELCEFYSRDPDGLPCNLRKPCNRPSGLEPQPGVFDCLRDAMVRDYVRQTWKLEGEALEQAIISQAPQVEKLIATTAHERMPWYHSSLTREEAERKLYSGAQTDGKFLLRPRKEQGTYALSLIYGKTVYHYLISQDKAGKYCIPEGTKFDTLWQLVEYLKLKADGLIYCLKEACPNSSASNASGGGSRRHQGKQNELSDTAGREINLVDAHLKSEQTEASTRQNSQVLLSETGIYDNDPDLCFRMQEGSEVYSNPCLEENKPGIVYASLNHSVIGPNSRLARNVKEAPTEYASICVRSSGGGSDEMEECSQHLPGAGSSGDIMDYKDDDDKGSSGTGSGSGTSAPITAYAQQTRGLLGCIITSLTGRDKNQVEGEVQIVSTATQTFLATCINGVCWAVYHGAGTRTIASPKGPVIQMYTNVDQDLVGWPAPQGSRSLTPCTCGSSDLYLVTRHADVIPVRRRGDSRGSLLSPRPISYLKGSSGGPLLCPAGHAVGLFRAAVCTRGVAKAVDFIPVENLETTMRSPVFTDNSSPPAVTLTHPITKIDTKYIMTCMSADLEVVTSTWVLVGGVLAALAAYCLSTGCVVIVGRIVLSGKPAIIPDREVLY

SEQ ID NO: 25 - protein, 686 aa, Artificial Sequence
  chimeric
MPDPAAHLPFFYGSISRAEAEEHLKLAGMADGLFLLRQCLRSLGGYVLSLVHDVRFHHFPIERQLNGTYAIAGGKAHCGPAELCEFYSRDPDGLPCNLRKPCNRPSGLEPQPGVFDCLRDAMVRDYVRQTWKLEGEALEQAIISQAPQVEKLIATTAHERMPWYHSSLTREEAERKLYSGAQTDGKFLLRPRKEQGTYALSLIYGKTVYHYLISQDKAGKYCIPEGTKFDTLWQLVEYLKLKADGLIYCLKEACPNSSASNASGGGSRIRQKKAQGSTSSTRLHEPEKNAREITQDTNDITYADLNLPKGKKPAPQAAEPNNHTEYASIQTSPQPASEDTLTYADLDMVHLNRTPKQPAPKPEPSFSEYASVQVPRKSGGGSDEMEECSQHLPGAGSSGDIMDYKDDDDKGSSGTGSGSGTSAPITAYAQQTRGLLGCIITSLTGRDKNQVEGEVQIVSTATQTFLATCINGVCWAVYHGAGTRTIASPKGPVIQMYTNVDQDLVGWPAPQGSRSLTPCTCGSSDLYLVTRHADVIPVRRRGDSRGSLLSPRPISYLKGSSGGPLLCPAGHAVGLFRAAVCTRGVAKAVDFIPVENLETTMRSPVFTDNSSPPAVTLTHPITKIDTKYIMTCMSADLEVVTSTWVLVGGVLAALAAYCLSTGCVVIVGRIVLSGKPAIIPDREVLY

SEQ ID NO: 26 - protein, 665 aa, Artificial Sequence
  chimeric
MPDPAAHLPFFYGSISRAEAEEHLKLAGMADGLFLLRQCLRSLGGYVLSLVHDVRFHHFPIERQLNGTYAIAGGKAHCGPAELCEFYSRDPDGLPCNLRKPCNRPSGLEPQPGVFDCLRDAMVRDYVRQTWKLEGEALEQAIISQAPQVEKLIATTAHERMPWYHSSLTREEAERKLYSGAQTDGKFLLRPRKEQGTYALSLIYGKTVYHYLISQDKAGKYCIPEGTKFDTLWQLVEYLKLKADGLIYCLKEACPNSSASNASGGGSKARRKQAAGRPEKMDDEDPIMGTITSGSRKKPWPDSPGDQASPPGDAPPLEEQKELHYASLSFSEMKSREPKDQEAPSTTEYSEIKTSKSGGGSDEMEECSQHLPGAGSSGDIMDYKDDDDKGSSGTGSGSGTSAPITAYAQQTRGLLGCIITSLTGRDKNQVEGEVQIVSTATQTFLATCINGVCWAVYHGAGTRTIASPKGPVIQMYTNVDQDLVGWPAPQGSRSLTPCTCGSSDLYLVTRHADVIPVRRRGDSRGSLLSPRPISYLKGSSGGPLLCPAGHAVGLFRAAVCTRGVAKAVDFIPVENLETTMRSPVFTDNSSPPAVTLTHPITKIDTKYIMTCMSADLEVVTSTWVLVGGVLAALAAYCLSTGCVVIVGRIVLSGKPAIIPDREVLY

SEQ ID NO: 27 - protein, 670 aa, Artificial Sequence
  chimeric
MPDPAAHLPFFYGSISRAEAEEHLKLAGMADGLFLLRQCLRSLGGYVLSLVHDVRFHHFPIERQLNGTYAIAGGKAHCGPAELCEFYSRDPDGLPCNLRKPCNRPSGLEPQPGVFDCLRDAMVRDYVRQTWKLEGEALEQAIISQAPQVEKLIATTAHERMPWYHSSLTREEAERKLYSGAQTDGKFLLRPRKEQGTYALSLIYGKTVYHYLISQDKAGKYCIPEGTKFDTLWQLVEYLKLKADGLIYCLKEACPNSSASNASGGGSVRSCRKKSARPAAGVGDTGIEDANAVRGSASQGPLTEPWAEDSPPDQPPPASARSSVGEGELQYASLSFQMVKPWDSRGQEATDTEYSEIKIHRSGGGSDEMEECSQHLPGAGSSGDIMDYKDDDDKGSSGTGSGSGTSAPITAYAQQTRGLLGCIITSLTGRDKNQVEGEVQIVSTATQTFLATCINGVCWAVYHGAGTRTIASPKGPVIQMYTNVDQDLVGWPAPQGSRSLTPCTCGSSDLYLVTRHADVIPVRRRGDSRGSLLSPRPISYLKGSSGGPLLCPAGHAVGLFRAAVCTRGVAKAVDFIPVENLETTMRSPVFTDNSSPPAVTLTHPITKIDTKYIMTCMSADLEVVTSTWVLVGGVLAALAAYCLSTGCVVIVGRIVLSGKPAIIPDREVLY

SEQ ID NO: 28 - protein, 690 aa, Artificial Sequence
  chimeric
MPDPAAHLPFFYGSISRAEAEEHLKLAGMADGLFLLRQCLRSLGGYVLSLVHDVRFHHFPIERQLNGTYAIAGGKAHCGPAELCEFYSRDPDGLPCNLRKPCNRPSGLEPQPGVFDCLRDAMVRDYVRQTWKLEGEALEQAIISQAPQVEKLIATTAHERMPWYHSSLTREEAERKLYSGAQTDGKFLLRPRKEQGTYALSLIYGKTVYHYLISQDKAGKYCIPEGTKFDTLWQLVEYLKLKADGLIYCLKEACPNSSASNASGGGSKICRKEARKRAAAEQDVPSTLGPISQGHQHECSAGSSQDHPPPGAATYTPGKGEEQELHYASLSFQGLRLWEPADQEAPSTTEYSEIKIHTGQPLRGPGFGLQLEREMSGMVPKSGGGSDEMEECSQHLPGAGSSGDIMDYKDDDDKGSSGTGSGSGTSAPITAYAQQTRGLLGCIITSLTGRDKNQVEGEVQIVSTATQTFLATCINGVCWAVYHGAGTRTIASPKGPVIQMYTNVDQDLVGWPAPQGSRSLTPCTCGSSDLYLVTRHADVIPVRRRGDSRGSLLSPRPISYLKGSSGGPLLCPAGHAVGLFRAAVCTRGVAKAVDFIPVENLETTMRSPVFTDNSSPPAVTLTHPITKIDTKYIMTCMSADLEVVTSTWVLVGGVLAALAAYCLSTGCVVIVGRIVLSGKPAIIPDREVLY

SEQ ID NO: 29 - protein, 694 aa, Artificial Sequence
  chimeric
MPDPAAHLPFFYGSISRAEAEEHLKLAGMADGLFLLRQCLRSLGGYVLSLVHDVRFHHFPIERQLNGTYAIAGGKAHCGPAELCEFYSRDPDGLPCNLRKPCNRPSGLEPQPGVFDCLRDAMVRDYVRQTWKLEGEALEQAIISQAPQVEKLIATTAHERMPWYHSSLTREEAERKLYSGAQTDGKFLLRPRKEQGTYALSLIYGKTVYHYLISQDKAGKYCIPEGTKFDTLWQLVEYLKLKADGLIYCLKEACPNSSASNASGGGSKCYFLRKAKAKQMPVEMSRPAVPLLNSNNEKMSDPNMEANSHYGHNDDVRNHAMKPINDNKEPLNSDVQYTEVQVSSAESHKDLGKKDTETVYSEVRKAVPDAVESRYSRTEGSLDGTSGGGSDEMEECSQHLPGAGSSGDIMDYKDDDDKGSSGTGSGSGTSAPITAYAQQTRGLLGCIITSLTGRDKNQVEGEVQIVSTATQTFLATCINGVCWAVYHGAGTRTIASPKGPVIQMYTNVDQDLVGWPAPQGSRSLTPCTCGSSDLYLVTRHADVIPVRRRGDSRGSLLSPRPISYLKGSSGGPLLCPAGHAVGLFRAAVCTRGVAKAVDFIPVENLETTMRSPVFTDNSSPPAVTLTHPITKIDTKYIMTCMSADLEVVTSTWVLVGGVLAALAAYCLSTGCVVIVGRIVLSGKPAIIPDREVLY

SEQ ID NO: 30 - protein, 755 aa, Artificial Sequence
  chimeric
MPDPAAHLPFFYGSISRAEAEEHLKLAGMADGLFLLRQCLRSLGGYVLSLVHDVRFHHFPIERQLNGTYAIAGGKAHCGPAELCEFYSRDPDGLPCNLRKPCNRPSGLEPQPGVFDCLRDAMVRDYVRQTWKLEGEALEQAIISQAPQVEKLIATTAHERMPWYHSSLTREEAERKLYSGAQTDGKFLLRPRKEQGTYALSLIYGKTVYHYLISQDKAGKYCIPEGTKFDTLWQLVEYLKLKADGLIYCLKEACPNSSASNASGGGSKRKGRCSVPAFCSSQAEAPADTPEPTAGHTLYSVLSQGYEKLDTPLRPARQQPTPTSDSSSDSNLTTEEDEDRPEVHKPISGRYEVFDQVTQEGAGHDPAPEGQADYDPVTPYVTEVESVVGENTMYAQVFNLQGKTPVSQKEESSATIYCSIRKPQVVPPPQQNDLEIPESPTYENFTSGGGSDEMEECSQHLPGAGSSGDIMDYKDDDDKGSSGTGSGSGTSAPITAYAQQTRGLLGCIITSLTGRDKNQVEGEVQIVSTATQTFLATCINGVCWAVYHGAGTRTIASPKGPVIQMYTNVDQDLVGWPAPQGSRSLTPCTCGSSDLYLVTRHADVIPVRRRGDSRGSLLSPRPISYLKGSSGGPLLCPAGHAVGLFRAAVCTRGVAKAVDFIPVENLETTMRSPVFTDNSSPPAVTLTHPITKIDTKYIMTCMSADLEVVTSTWVLVGGVLAALAAYCLSTGCVVIVGRIVLSGKPAIIPDREVLY

SEQ ID NO: 31 - protein, 476 aa, Artificial Sequence
  chimeric
MPDPAAHLPFFYGSISRAEAEEHLKLAGMADGLFLLRQCLRSLGGYVLSLVHDVRFHHFPIERQLNGTYAIAGGKAHCGPAELCEFYSRDPDGLPCNLRKPCNRPSGLEPQPGVFDCLRDAMVRDYVRQTWKLEGEALEQAIISQAPQVEKLIATTAHERMPWYHSSLTREEAERKLYSGAQTDGKFLLRPRKEQGTYALSLIYGKTVYHYLISQDKAGKYCIPEGTKFDTLWQLVEYLKLKADGLIYCLKEACPNSSASNASGGGSCSRAARGTIGARRTGQPLKEDPSAVPVFSVDYGELDFQWREKTPEPPVPCVPEQTEYATIVFPSGMGTSSPARRGSADGPRSAQPLRPEDGHCSWPLSGGGSGVQVETISPGDGRTFPKRGQTCVVHYTGMLEDGKKVDSSRDRNKPFKFMLGKQEVIRGWEEGVAQMSVGQRAKLTISPDYAYGATGHPGIIPPHATLVFDVELLKLE

SEQ ID NO: 32 - protein, 696 aa, Artificial Sequence
  chimeric
MASSGMADSANHLPFFFGNITREEAEDYLVQGGMSDGLYLLRQSRNYLGGFALSVAHGRKAHHYTIERELNGTYAIAGGRTHASPADLCHYHSQESDGLVCLLKKPFNRPQGVQPKTGPFEDLKENLIREYVKQTWNLQGQALEQAIISQKPQLEKLIATTAHEKMPWFHGKISREESEQIVLIGSKTNGKFLIRARDNNGSYALCLLHEGKVLHYRIDKDKTGKLSIPEGKKFDTLWQLVEHYSYKADGLLRVLTVPCQKIGTQGNVNFGGRPQLPGSHPATWSAGGGSCSRAARGTIGARRTGQPLKEDPSAVPVFSVDYGELDFQWREKTPEPPVPCVPEQTEYATIVFPSGMGTSSPARRGSADGPRSAQPLRPEDGHCSWPLSGGGSDEMEECSQHLPGAGSSGDIMDYKDDDDKGSSGTGSGSGTSAPITAYAQQTRGLLGCIITSLTGRDKNQVEGEVQIVSTATQTFLATCINGVCWAVYHGAGTRTIASPKGPVIQMYTNVDQDLVGWPAPQGSRSLTPCTCGSSDLYLVTRHADVIPVRRRGDSRGSLLSPRPISYLKGSSGGPLLCPAGHAVGLFRAAVCTRGVAKAVDFIPVENLETTMRSPVFTDNSSPPAVTLTHPITKIDTKYIMTCMSADLEVVTSTWVLVGGVLAALAAYCLSTGCVVIVGRIVLSGKPAIIPDREVLY

SEQ ID NO: 33 - protein, 663 aa, Artificial Sequence
  chimeric
MGCGCSSHPEDDWMENIDVCENCHYPIVPLDGKGTLLIRNGSEVRDPLVTYEGSNPPASPLQDNLVIALHSYEPSHDGDLGFEKGEQLRILEQSGEWWKAQSLTTGQEGFIPFNFVAKANSLEPEPWFFKNLSRKDAERQLLAPGNTHGSFLIRESESTAGSFSLSVRDFDQNQGEVVKHYKIRNLDNGGFYISPRITFPGLHELVRHYTNASDGLCTRLSRPCQTQKPQKPWWEDEWEVPRETLKLVERLGAGGGSCSRAARGTIGARRTGQPLKEDPSAVPVFSVDYGELDFQWREKTPEPPVPCVPEQTEYATIVFPSGMGTSSPARRGSADGPRSAQPLRPEDGHCSWPLSGGGSDEMEECSQHLPGAGSSGDIMDYKDDDDKGSSGTGSGSGTSAPITAYAQQTRGLLGCIITSLTGRDKNQVEGEVQIVSTATQTFLATCINGVCWAVYHGAGTRTIASPKGPVIQMYTNVDQDLVGWPAPQGSRSLTPCTCGSSDLYLVTRHADVIPVRRRGDSRGSLLSPRPISYLKGSSGGPLLCPAGHAVGLFRAAVCTRGVAKAVDFIPVENLETTMRSPVFTDNSSPPAVTLTHPITKIDTKYIMTCMSADLEVVTSTWVLVGGVLAALAAYCLSTGCVVIVGRIVLSGKPAIIPDREVLY

SEQ ID NO: 34 - protein, 573 aa, Artificial Sequence
  chimeric
MPDPAAHLPFFYGSISRAEAEEHLKLAGMADGLFLLRQCLRSLGGYVLSLVHDVRFHHFPIERQLNGTYAIAGGKAHCGPAELCEFYSRDPDGLPCNLRKPCNRPSGLEPQPGVFDCLRDAMVRDYVRQTWKLEGEALEQAIISQAPQVEKLIATTAHERMPWYHSSLTREEAERKLYSGAQTDGKFLLRPRKEQGTYALSLIYGKTVYHYLISQDKAGKYCIPEGTKFDTLWQLVEYLKLKADGLIYCLKEACPNSSASNASGSGGGSDEMEECSQHLPGAGSSGDIMDYKDDDDKGSSGTGSGSGTSAPITAYAQQTRGLLGCIITSLTGRDKNQVEGEVQIVSTATQTFLATCINGVCWAVYHGAGTRTIASPKGPVIQMYTNVDQDLVGWPAPQGSRSLTPCTCGSSDLYLVTRHADVIPVRRRGDSRGSLLSPRPISYLKGSSGGPLLCPAGHAVGLFRAAVCTRGVAKAVDFIPVENLETTMRSPVFTDNSSPPAVTLTHPITKIDTKYIMTCMSADLEVVTSTWVLVGGVLAALAAYCLSTGCVVIVGRIVLSGKPAIIPDREVLY

SEQ ID NO: 35 - protein, 107 aa, Artificial Sequence
  Artificial
GVQVETISPGDGRTFPKRGQTCVVHYTGMLEDGKKVDSSRDRNKPFKFMLGKQEVIRGWEEGVAQMSVGQRAKLTISPDYAYGATGHPGIIPPHATLVFDVELLKLE

SEQ ID NO: 36 - protein, 674 aa, Artificial Sequence
  artifical
MAPDPAAHLPFFYGSISRAEAEEHLKLAGMADGLFLLRQCLRSLGGYVLSLVHDVRFHHFPIERQLNGTYAIAGGKAHCGPAELCEFYSRDPDGLPCNLRKPCNRPSGLEPQPGVFDCLRDAMVRDYVRQTWKLEGEALEQAIISQAPQVEKLIATTAHERMPWYHSSLTREEAERKLYSGAQTDGKFLLRPRKEQGTYALSLIYGKTVYHYLISQDKAGKYCIPEGTKFDTLWQLVEYLKLKADGLIYCLKEACPNSSASNASGGGSCSRAARGTIGARRTGQPLKEDPSAVPVFSVDYGELDFQWREKTPEPPVPCVPEQTEYATIVFPSGMGTSSPARRGSADGPRSAQPLRPEDGHCSWPLSGGGSDEMEECSQHLPGAGSSGDIMDYKDDDDKGSSGTGSGSGTSAPITAYAQQTRGLLGCIITSLTGRDKNQVEGEVQIVSTATQTFLATCINGVCWAVYHGAGTRTIASPKGPVIQMYTNVDQDLVGWPAPQGSRSLTPCTCGSSDLYLVTRHADVIPVRRRGDSRGSLLSPRPISYLKGSSGGPLLCPAGHAVGLFRAAVCTRGVAKAVDFIPVENLETTMRSPVFTDNSSPPAVTLTHPITKIDTKYIMTCMSADLEVVTSTWVLVGGVLAALAAYCLSTGCVVIVGRIVLSGKPAIIPDREVLY

SEQ ID NO: 37 - protein, 619 aa, Artificial Sequence
  artificial
MPDPAAHLPFFYGSISRAEAEEHLKLAGMADGLFLLRQCLRSLGGYVLSLVHDVRFHHFPIERQLNGTYAIAGGKAHCGPAELCEFYSRDPDGLPCNLRKPCNRPSGLEPQPGVFDCLRDAMVRDYVRQTWKLEGEALEQAIISQAPQVEKLIATTAHERMPWYHSSLTREEAERKLYSGAQTDGKFLLRPRKEQGTYALSLIYGKTVYHYLISQDKAGKYCIPEGTKFDTLWQLVEYLKLKADGLIYCLKEACPNSSASNASGAAAPTLPAHPSTLTHPQRRIDTLNSDGYTPEPARITSPDKPRPMPMDTSVYESPYSDPEELKDKKLFLKRDNLLIADIELGCGNFGSVRQGVYRMRKKQIDVAIKVLKQGTEKADTEEMMREAQIMHQLDNPYIVRLIGVCQAEALMLVMEMAGGGPLHKFLVGKREEIPVSNVAELLHQVSMGMKYLEEKNFVHRDLAARNVLLVNRHYAKISDFGLSKALGADDSYYTARSAGKWPLKWYAPECINFRKFSSRSDVWSYGVTMWEALSYGQKPYKKMKGPEVMAFIEQGKRMECPPECPPELYALMSDCWIYKWEDRPDFLTVEQRMRACYYSLASKVEGPPGSTQKAEAACA

SEQ ID NO: 38 - protein, 635 aa, Artificial Sequence
  artificial
MASSGMADSANHLPFFFGNITREEAEDYLVQGGMSDGLYLLRQSRNYLGGFALSVAHGRKAHHYTIERELNGTYAIAGGRTHASPADLCHYHSQESDGLVCLLKKPFNRPQGVQPKTGPFEDLKENLIREYVKQTWNLQGQALEQAIISQKPQLEKLIATTAHEKMPWFHGKISREESEQIVLIGSKTNGKFLIRARDNNGSYALCLLHEGKVLHYRIDKDKTGKLSIPEGKKFDTLWQLVEHYSYKADGLLRVLTVPCQKIGTQGNVNFGGRPQLPGSHPATWSAGGIISRIKSYSFPKPGHRKSSPAQGNRQESTVSFNPYEPELAPWAADKGPQREALPMDTEVYESPYADPEEIRPKEVYLDRKLLTLEDKELGSGNFGTVKKGYYQMKKVVKTVAVKILKNEANDPALKDELLAEANVMQQLDNPYIVRMIGICEAESWMLVMEMAELGPLNKYLQQNRHVKDKNIIELVHQVSMGMKYLEESNFVHRDLAARNVLLVTQHYAKISDFGLSKALRADENYYKAQTHGKWPVKWYAPECINYYKFSSKSDVWSFGVLMWEAFSYGQKPYRGMKGSEVTAMLEKGERMGCPAGCPREMYDLMNLCWTYDVENRPGFAAVELRLRNYYYDVVN

SEQ ID NO: 39 - protein, 509 aa, Artificial Sequence
  artifical
MGCGCSSHPEDDWMENIDVCENCHYPIVPLDGKGTLLIRNGSEVRDPLVTYEGSNPPASPLQDNLVIALHSYEPSHDGDLGFEKGEQLRILEQSGEWWKAQSLTTGQEGFIPFNFVAKANSLEPEPWFFKNLSRKDAERQLLAPGNTHGSFLIRESESTAGSFSLSVRDFDQNQGEVVKHYKIRNLDNGGFYISPRITFPGLHELVRHYTNASDGLCTRLSRPCQTQKPQKPWWEDEWEVPRETLKLVERLGAGQFGEVWMGYYNGHTKVAVKSLKQGSMSPDAFLAEANLMKQLQHQRLVRLYAVVTQEPIYIITEYMENGSLVDFLKTPSGIKLTINKLLDMAAQIAEGMAFIEERNYIHRDLRAANILVSDTLSCKIADFGLARLIEDNEYTAREGAKFPIKWTAPEAINYGTFTIKSDVWSFGILLTEIVTHGRIPYPGMTNPEVIQNLERGYRMVRPDNCPEELYQLMRLCWKERPEDRPTFDYLRSVLEDFFTATEGQYQPQP

SEQ ID NO: 40 - protein, 304 aa, Artificial Sequence
  artificial
DEMEECSQHLPGAGSSGDIMDYKDDDDKGSSGTGSGSGTSAPITAYAQQTRGLLGCIITSLTGRDKNQVEGEVQIVSTATQTFLATCINGVCWAVYHGAGTRTIASPKGPVIQMYTNVDQDLVGWPAPQGSRSLTPCTCGSSDLYLVTRHADVIPVRRRGDSRGSLLSPRPISYLKGSSGGPLLCPAGHAVGLFRAAVCTRGVAKAVDFIPVENLETTMRSPVFTDNSSPPAVTLTHPITKIDTKYIMTCMSADLEVVTSTWVLVGGVLAALAAYCLSTGCVVIVGRIVLSGKPAIIPDREVLY

SEQ ID NO: 41 - protein, 51 aa, Artificial Sequence
  IKZF1 ZF2-3
FQCNQCGASFTQKGNLLRHIKLHSGEKPFKCHLCNYACRRRDALTGHLRTH

SEQ ID NO: 42 - protein, 51 aa, Artificial Sequence
  42
FQCNQCGASFTQKGNLLRHIKLHTGEKPFKCHLCNYACQRRDALTGHLRTH

SEQ ID NO: 43 - protein, 54 aa, Artificial Sequence
  43
LQCEICGFTCRQKASLNWHMKKHDADSFYQFSCNICGKKFEKKDSVVAHKAKSH

SEQ ID NO: 44 - protein, 54 aa, Artificial Sequence
  44
LQCEVCGFQCRQRASLKYHMTKHKAETELDFACDQCGRRFEKAHNLNVHMSMVH

SEQ ID NO: 45 - protein, 54 aa, Artificial Sequence
  45
LQCEICGYQCRQRASLNWHMKKHTAEVQYNFTCDRCGKRFEKLDSVKFHTLKSH

SEQ ID NO: 46 - protein, 55 aa, Artificial Sequence
  46
LQCEICGFTCRQKASLNWHQRKHAETVAALRFPCEFCGKRFEKPDSVAAHRSKSH

SEQ ID NO: 47 - protein, 51 aa, Artificial Sequence
  47
LQCEICGFTCRQKGNLLRHIKLHSGEKPFKCHLCNYACRRRDALTGHLRTH

SEQ ID NO: 48 - protein, 23 aa, Artificial Sequence
  48
LQCEICGFTCRQKGNLLRHIKLH

SEQ ID NO: 49 - protein, 51 aa, Artificial Sequence
  49
LQCEICGYQCRQKGNLLRHIKLHSGEKPFKCHLCNYACRRRDALTGHLRTH

SEQ ID NO: 50 - protein, 51 aa, Artificial Sequence
  50
LQCEVCGFQCRQKGNLLRHIKLHSGEKPFKCHLCNYACRRRDALTGHLRTH

SEQ ID NO: 51 - protein, 51 aa, Artificial Sequence
  51
FQCPICGLVIKQKGNLLRHIKLHSGEKPFKCHLCNYACRRRDALTGHLRTH

SEQ ID NO: 52 - protein, 11 aa, Artificial Sequence
  52
LQCEICGFTCR

SEQ ID NO: 53 - protein, 11 aa, Artificial Sequence
  53
LQCEICGYQCR

SEQ ID NO: 54 - protein, 11 aa, Artificial Sequence
  54
LQCEVCGFQCR

SEQ ID NO: 55 - protein, 11 aa, Artificial Sequence
  55
FQCPICGLVIK

SEQ ID NO: 56 - protein, 12 aa, Artificial Sequence
  56
QKGNLLRHIKLH

SEQ ID NO: 57 - protein, 23 aa, Artificial Sequence
  57
FKCHLCNYACRRRDALTGHLRTH

SEQ ID NO: 58 - protein, 426 aa, Artificial Sequence
  58
MPDPAAHLPFFYGSISRAEAEEHLKLAGMADGLFLLRQCLRSLGGYVLSLVHDVRFHHFPIERQLNGTYAIAGGKAHCGPAELCEFYSRDPDGLPCNLRKPCNRPSGLEPQPGVFDCLRDAMVRDYVRQTWKLEGEALEQAIISQAPQVEKLIATTAHERMPWYHSSLTREEAERKLYSGAQTDGKFLLRPRKEQGTYALSLIYGKTVYHYLISQDKAGKYCIPEGTKFDTLWQLVEYLKLKADGLIYCLKEACPNSSASNASGGGSCSRAARGTIGARRTGQPLKEDPSAVPVFSVDYGELDFQWREKTPEPPVPCVPEQTEYATIVFPSGMGTSSPARRGSADGPRSAQPLRPEDGHCSWPLSGGGSGERPFQCNQCGASFTQKGNLLRHIKLHSGEKPFKCHLCNYACRRRDALTGHLRTHSV

SEQ ID NO: 59 - protein, 426 aa, Artificial Sequence
  59
MPDPAAHLPFFYGSISRAEAEEHLKLAGMADGLFLLRQCLRSLGGYVLSLVHDVRFHHFPIERQLNGTYAIAGGKAHCGPAELCEFYSRDPDGLPCNLRKPCNRPSGLEPQPGVFDCLRDAMVRDYVRQTWKLEGEALEQAIISQAPQVEKLIATTAHERMPWYHSSLTREEAERKLYSGAQTDGKFLLRPRKEQGTYALSLIYGKTVYHYLISQDKAGKYCIPEGTKFDTLWQLVEYLKLKADGLIYCLKEACPNSSASNASGGGSCSRAARGTIGARRTGQPLKEDPSAVPVFSVDYGELDFQWREKTPEPPVPCVPEQTEYATIVFPSGMGTSSPARRGSADGPRSAQPLRPEDGHCSWPLSGGGSGERPFQCNQCGASFTQKGNLLRHIKLHTGEKPFKCHLCNYACQRRDALTGHLRTHSV

SEQ ID NO: 60 - protein, 429 aa, Artificial Sequence
  60
MPDPAAHLPFFYGSISRAEAEEHLKLAGMADGLFLLRQCLRSLGGYVLSLVHDVRFHHFPIERQLNGTYAIAGGKAHCGPAELCEFYSRDPDGLPCNLRKPCNRPSGLEPQPGVFDCLRDAMVRDYVRQTWKLEGEALEQAIISQAPQVEKLIATTAHERMPWYHSSLTREEAERKLYSGAQTDGKFLLRPRKEQGTYALSLIYGKTVYHYLISQDKAGKYCIPEGTKFDTLWQLVEYLKLKADGLIYCLKEACPNSSASNASGGGSCSRAARGTIGARRTGQPLKEDPSAVPVFSVDYGELDFQWREKTPEPPVPCVPEQTEYATIVFPSGMGTSSPARRGSADGPRSAQPLRPEDGHCSWPLSGGGSGEKPLQCEICGFTCRQKASLNWHMKKHDADSFYQFSCNICGKKFEKKDSVVAHKAKSHPE

SEQ ID NO: 61 - protein, 429 aa, Artificial Sequence
  61
MPDPAAHLPFFYGSISRAEAEEHLKLAGMADGLFLLRQCLRSLGGYVLSLVHDVRFHHFPIERQLNGTYAIAGGKAHCGPAELCEFYSRDPDGLPCNLRKPCNRPSGLEPQPGVFDCLRDAMVRDYVRQTWKLEGEALEQAIISQAPQVEKLIATTAHERMPWYHSSLTREEAERKLYSGAQTDGKFLLRPRKEQGTYALSLIYGKTVYHYLISQDKAGKYCIPEGTKFDTLWQLVEYLKLKADGLIYCLKEACPNSSASNASGGGSCSRAARGTIGARRTGQPLKEDPSAVPVFSVDYGELDFQWREKTPEPPVPCVPEQTEYATIVFPSGMGTSSPARRGSADGPRSAQPLRPEDGHCSWPLSGGGSGAKPLQCEVCGFQCRQRASLKYHMTKHKAETELDFACDQCGRRFEKAHNLNVHMSMVHPL

SEQ ID NO: 62 - protein, 429 aa, Artificial Sequence
  62
MPDPAAHLPFFYGSISRAEAEEHLKLAGMADGLFLLRQCLRSLGGYVLSLVHDVRFHHFPIERQLNGTYAIAGGKAHCGPAELCEFYSRDPDGLPCNLRKPCNRPSGLEPQPGVFDCLRDAMVRDYVRQTWKLEGEALEQAIISQAPQVEKLIATTAHERMPWYHSSLTREEAERKLYSGAQTDGKFLLRPRKEQGTYALSLIYGKTVYHYLISQDKAGKYCIPEGTKFDTLWQLVEYLKLKADGLIYCLKEACPNSSASNASGGGSCSRAARGTIGARRTGQPLKEDPSAVPVFSVDYGELDFQWREKTPEPPVPCVPEQTEYATIVFPSGMGTSSPARRGSADGPRSAQPLRPEDGHCSWPLSGGGSGETPLQCEICGYQCRQRASLNWHMKKHTAEVQYNFTCDRCGKRFEKLDSVKFHTLKSHPD

SEQ ID NO: 63 - protein, 430 aa, Artificial Sequence
  63
MPDPAAHLPFFYGSISRAEAEEHLKLAGMADGLFLLRQCLRSLGGYVLSLVHDVRFHHFPIERQLNGTYAIAGGKAHCGPAELCEFYSRDPDGLPCNLRKPCNRPSGLEPQPGVFDCLRDAMVRDYVRQTWKLEGEALEQAIISQAPQVEKLIATTAHERMPWYHSSLTREEAERKLYSGAQTDGKFLLRPRKEQGTYALSLIYGKTVYHYLISQDKAGKYCIPEGTKFDTLWQLVEYLKLKADGLIYCLKEACPNSSASNASGGGSCSRAARGTIGARRTGQPLKEDPSAVPVFSVDYGELDFQWREKTPEPPVPCVPEQTEYATIVFPSGMGTSSPARRGSADGPRSAQPLRPEDGHCSWPLSGGGSGEKPLQCEICGFTCRQKASLNWHQRKHAETVAALRFPCEFCGKRFEKPDSVAAHRSKSHPA

SEQ ID NO: 64 - protein, 398 aa, Artificial Sequence
  64
MPDPAAHLPFFYGSISRAEAEEHLKLAGMADGLFLLRQCLRSLGGYVLSLVHDVRFHHFPIERQLNGTYAIAGGKAHCGPAELCEFYSRDPDGLPCNLRKPCNRPSGLEPQPGVFDCLRDAMVRDYVRQTWKLEGEALEQAIISQAPQVEKLIATTAHERMPWYHSSLTREEAERKLYSGAQTDGKFLLRPRKEQGTYALSLIYGKTVYHYLISQDKAGKYCIPEGTKFDTLWQLVEYLKLKADGLIYCLKEACPNSSASNASGGGSCSRAARGTIGARRTGQPLKEDPSAVPVFSVDYGELDFQWREKTPEPPVPCVPEQTEYATIVFPSGMGTSSPARRGSADGPRSAQPLRPEDGHCSWPLSGGGSGERPLQCEICGFTCRQKGNLLRHIKLHSG

SEQ ID NO: 65 - protein, 426 aa, Artificial Sequence
  65
MPDPAAHLPFFYGSISRAEAEEHLKLAGMADGLFLLRQCLRSLGGYVLSLVHDVRFHHFPIERQLNGTYAIAGGKAHCGPAELCEFYSRDPDGLPCNLRKPCNRPSGLEPQPGVFDCLRDAMVRDYVRQTWKLEGEALEQAIISQAPQVEKLIATTAHERMPWYHSSLTREEAERKLYSGAQTDGKFLLRPRKEQGTYALSLIYGKTVYHYLISQDKAGKYCIPEGTKFDTLWQLVEYLKLKADGLIYCLKEACPNSSASNASGGGSCSRAARGTIGARRTGQPLKEDPSAVPVFSVDYGELDFQWREKTPEPPVPCVPEQTEYATIVFPSGMGTSSPARRGSADGPRSAQPLRPEDGHCSWPLSGGGSGERPLQCEICGYQCRQKGNLLRHIKLHSGEKPFKCHLCNYACRRRDALTGHLRTHSV

SEQ ID NO: 66 - protein, 426 aa, Artificial Sequence
  66
MPDPAAHLPFFYGSISRAEAEEHLKLAGMADGLFLLRQCLRSLGGYVLSLVHDVRFHHFPIERQLNGTYAIAGGKAHCGPAELCEFYSRDPDGLPCNLRKPCNRPSGLEPQPGVFDCLRDAMVRDYVRQTWKLEGEALEQAIISQAPQVEKLIATTAHERMPWYHSSLTREEAERKLYSGAQTDGKFLLRPRKEQGTYALSLIYGKTVYHYLISQDKAGKYCIPEGTKFDTLWQLVEYLKLKADGLIYCLKEACPNSSASNASGGGSCSRAARGTIGARRTGQPLKEDPSAVPVFSVDYGELDFQWREKTPEPPVPCVPEQTEYATIVFPSGMGTSSPARRGSADGPRSAQPLRPEDGHCSWPLSGGGSGERPLQCEICGFTCRQKGNLLRHIKLHSGEKPFKCHLCNYACRRRDALTGHLRTHSV

SEQ ID NO: 67 - protein, 426 aa, Artificial Sequence
  67
MPDPAAHLPFFYGSISRAEAEEHLKLAGMADGLFLLRQCLRSLGGYVLSLVHDVRFHHFPIERQLNGTYAIAGGKAHCGPAELCEFYSRDPDGLPCNLRKPCNRPSGLEPQPGVFDCLRDAMVRDYVRQTWKLEGEALEQAIISQAPQVEKLIATTAHERMPWYHSSLTREEAERKLYSGAQTDGKFLLRPRKEQGTYALSLIYGKTVYHYLISQDKAGKYCIPEGTKFDTLWQLVEYLKLKADGLIYCLKEACPNSSASNASGGGSCSRAARGTIGARRTGQPLKEDPSAVPVFSVDYGELDFQWREKTPEPPVPCVPEQTEYATIVFPSGMGTSSPARRGSADGPRSAQPLRPEDGHCSWPLSGGGSGERPLQCEVCGFQCRQKGNLLRHIKLHSGEKPFKCHLCNYACRRRDALTGHLRTHSV

SEQ ID NO: 68 - protein, 426 aa, Artificial Sequence
  68
MPDPAAHLPFFYGSISRAEAEEHLKLAGMADGLFLLRQCLRSLGGYVLSLVHDVRFHHFPIERQLNGTYAIAGGKAHCGPAELCEFYSRDPDGLPCNLRKPCNRPSGLEPQPGVFDCLRDAMVRDYVRQTWKLEGEALEQAIISQAPQVEKLIATTAHERMPWYHSSLTREEAERKLYSGAQTDGKFLLRPRKEQGTYALSLIYGKTVYHYLISQDKAGKYCIPEGTKFDTLWQLVEYLKLKADGLIYCLKEACPNSSASNASGGGSCSRAARGTIGARRTGQPLKEDPSAVPVFSVDYGELDFQWREKTPEPPVPCVPEQTEYATIVFPSGMGTSSPARRGSADGPRSAQPLRPEDGHCSWPLSGGGSGERPFQCPICGLVIKQKGNLLRHIKLHSGEKPFKCHLCNYACRRRDALTGHLRTHSV